European Patent Application EP 4 702 991 A1, published March 4, 2026. Title: ANTIBODY-DRUG CONJUGATE. Applicant: CSPC Megalith Biopharmaceutical Co., Ltd. Application CN. The sequence listing filed with the application follows.

SEQUENCE LISTING (80 sequences)

SEQ ID NO: 1 - protein, 450 aa, synthetic construct
EVQLVESGGGLVQPGGSLRLSCAASGFNIKDTYIHWVRQAPGKGLEWVARIYPTNGYTRYADSVKGRFTISADTSKNTAYLQMNSLRAEDTAVYYCSRWGGDGFYAMDYWGQGTLVTVSSASTKGPSVFPLAPSSKSTSGGTAALGCLVKDYFPEPVTVSWNSGALTSGVHTFPAVLQSSGLYSLSSVVTVPSSSLGTQTYICNVNHKPSNTKVDKKVEPKSCDKTHTCPPCPAPELLGGPSVFLFPPKPKDTLMISRTPEVTCVVVDVSHEDPEVKFNWYVDGVEVHNAKTKPREEQYNSTYRVVSVLTVLHQDWLNGKEYKCKVSNKALPAPIEKTISKAKGQPREPQVYTLPPSREEMTKNQVSLTCLVKGFYPSDIAVEWESNGQPENNYKTTPPVLDSDGSFFLYSKLTVDKSRWQQGNVFSCSVMHEALHNHYTQKSLSLSPGK

SEQ ID NO: 2 - protein, 214 aa, synthetic construct
DIQMTQSPSSLSASVGDRVTITCRASQDVNTAVAWYQQKPGKAPKLLIYSASFLYSGVPSRFSGSRSGTDFTLTISSLQPEDFATYYCQQHYTTPPTFGQGTKVEIKRTVAAPSVFIFPPSDEQLKSGTASVVCLLNNFYPREAKVQWKVDNALQSGNSQESVTEQDSKDSTYSLSSTLTLSKADYEKHKVYACEVTHQGLSSPVTKSFNRGEC

SEQ ID NO: 3 - protein, 448 aa, synthetic construct
EVQLVESGGGLVQPGGSLRLSCAASGFTFTDYTMDWVRQAPGKGLEWVADVNPNSGGSIYNQRFKGRFTLSVDRSKNTLYLQMNSLRAEDTAVYYCARNLGPSFYFDYWGQGTLVTVSSASTKGPSVFPLAPSSKSTSGGTAALGCLVKDYFPEPVTVSWNSGALTSGVHTFPAVLQSSGLYSLSSVVTVPSSSLGTQTYICNVNHKPSNTKVDKKVEPKSCDKTHTCPPCPAPELLGGPSVFLFPPKPKDTLMISRTPEVTCVVVDVSHEDPEVKFNWYVDGVEVHNAKTKPREEQYNSTYRVVSVLTVLHQDWLNGKEYKCKVSNKALPAPIEKTISKAKGQPREPQVYTLPPSREEMTKNQVSLTCLVKGFYPSDIAVEWESNGQPENNYKTTPPVLDSDGSFFLYSKLTVDKSRWQQGNVFSCSVMHEALHNHYTQKSLSLSPG

SEQ ID NO: 4 - protein, 214 aa, synthetic construct
DIQMTQSPSSLSASVGDRVTITCKASQDVSIGVAWYQQKPGKAPKLLIYSASYRYTGVPSRFSGSGSGTDFTLTISSLQPEDFATYYCQQYYIYPYTFGQGTKVEIKRTVAAPSVFIFPPSDEQLKSGTASVVCLLNNFYPREAKVQWKVDNALQSGNSQESVTEQDSKDSTYSLSSTLTLSKADYEKHKVYACEVTHQGLSSPVTKSFNRGEC

SEQ ID NO: 5 - protein, 443 aa, synthetic construct
EVQLVQSGAEVKKPGSSVKVSCKASGYTITDSNIHWVRQAPGQSLEWIGYIYPYNGGTDYNQKFKNRATLTVDNPTNTAYMELSSLRSEDTAFYYCVNGNPWLAYWGQGTLVTVSSASTKGPSVFPLAPCSRSTSESTAALGCLVKDYFPEPVTVSWNSGALTSGVHTFPAVLQSSGLYSLSSVVTVPSSSLGTKTYTCNVDHKPSNTKVDKRVESKYGPPCPPCPAPEFLGGPSVFLFPPKPKDTLMISRTPEVTCVVVDVSQEDPEVQFNWYVDGVEVHNAKTKPREEQFNSTYRVVSVLTVLHQDWLNGKEYKCKVSNKGLPSSIEKTISKAKGQPREPQVYTLPPSQEEMTKNQVSLTCLVKGFYPSDIAVEWESNGQPENNYKTTPPVLDSDGSFFLYSRLTVDKSRWQEGNVFSCSVMHEALHNHYTQKSLSLSLGK

SEQ ID NO: 6 - protein, 218 aa, synthetic construct
DIQLTQSPSTLSASVGDRVTITCRASESLDNYGIRFLTWFQQKPGKAPKLLMYAASNQGSGVPSRFSGSGSGTEFTLTISSLQPDDFATYYCQQTKEVPWSFGQGTKVEVKRTVAAPSVFIFPPSDEQLKSGTASVVCLLNNFYPREAKVQWKVDNALQSGNSQESVTEQDSKDSTYSLSSTLTLSKADYEKHKVYACEVTHQGLSSPVTKSFNRGEC

SEQ ID NO: 7 - protein, 446 aa, synthetic construct
EVQLVQSGAEVKKPGSSVKVSCKASGYTITDSNIHWVRQAPGQSLEWIGYIYPYNGGTDYNQKFKNRATLTVDNPTNTAYMELSSLRSEDTAFYYCVNGNPWLAYWGQGTLVTVSSASTKGPSVFPLAPSSKSTSGGTAALGCLVKDYFPEPVTVSWNSGALTSGVHTFPAVLQSSGLYSLSSVVTVPSSSLGTQTYICNVNHKPSNTKVDKKVEPKSCDKTHTCPPCPAPELLGGPSVFLFPPKPKDTLMISRTPEVTCVVVDVSHEDPEVKFNWYVDGVEVHNAKTKPREEQYASTYRVVSVLTVLHQDWLNGKEYKCKVSNKALPAPIEKTISKAKGQPREPQVYTLPPSRDELTKNQVSLTCLVKGFYPSDIAVEWESNGQPENNYKTTPPVLDSDGSFFLYSKLTVDKSRWQQGNVFSCSVMHEALHNHYTQKSLSLSPGK

SEQ ID NO: 8 - protein, 218 aa, synthetic construct; identical to SEQ ID NO: 6

SEQ ID NO: 9 - protein, 445 aa, synthetic construct
QVQLQQPGAEVVKPGASVKMSCKASGYTFTSYYIHWIKQTPGQGLEWVGVIYPGNDDISYNQKFQGKATLTADKSSTTAYMQLSSLTSEDSAVYYCAREVRLRYFDVWGQGTTVTVSSASTKGPSVFPLAPCSRSTSESTAALGCLVKDYFPEPVTVSWNSGALTSGVHTFPAVLQSSGLYSLSSVVTVPSSSLGTKTYTCNVDHKPSNTKVDKRVESKYGPPCPPCPAPEFLGGPSVFLFPPKPKDTLMISRTPEVTCVVVDVSQEDPEVQFNWYVDGVEVHNAKTKPREEQFNSTYRVVSVLTVLHQDWLNGKEYKCKVSNKGLPSSIEKTISKAKGQPREPQVYTLPPSQEEMTKNQVSLTCLVKGFYPSDIAVEWESNGQPENNYKTTPPVLDSDGSFFLYSRLTVDKSRWQEGNVFSCSVMHEALHNHYTQKSLSLSLGK

SEQ ID NO: 10 - protein, 219 aa, synthetic construct
EIVLTQSPGSLAVSPGERVTMSCKSSQSVFFSSSQKNYLAWYQQIPGQSPRLLIYWASTRESGVPDRFTGSGSGTDFTLTISSVQPEDLAIYYCHQYLSSRTFGQGTKLEIKRTVAAPSVFIFPPSDEQLKSGTASVVCLLNNFYPREAKVQWKVDNALQSGNSQESVTEQDSKDSTYSLSSTLTLSKADYEKHKVYACEVTHQGLSSPVTKSFNRGEC

SEQ ID NO: 11 - protein, 447 aa, synthetic construct
QVQLVQSGAEVKKPGASVKVSCKASGYTFTNYDINWVRQAPGQGLEWIGWIYPGDGSTKYNEKFKAKATLTADTSTSTAYMELRSLRSDDTAVYYCASGYEDAMDYWGQGTTVTVSSASTKGPSVFPLAPSSKSTSGGTAALGCLVKDYFPEPVTVSWNSGALTSGVHTFPAVLQSSGLYSLSSVVTVPSSSLGTQTYICNVNHKPSNTKVDKKVEPKSCDKTHTCPPCPAPEAAGGPSVFLFPPKPKDTLMISRTPEVTCVVVDVSHEDPEVKFNWYVDGVEVHNAKTKPREEQYNSTYRVVSVLTVLHQDWLNGKEYKCKVSNKALAASIEKTISKAKGQPREPQVYTLPPSRDELTKNQVSLTCLVKGFYPSDIAVEWESNGQPENNYKTTPPVLDSDGSFFLYSKLTVDKSRWQQGNVFSCSVMHEALHNHYTQKSLSLSPGK

SEQ ID NO: 12 - protein, 214 aa, synthetic construct
DIQMTQSPSSLSASVGDRVTINCKASQDINSYLSWFQQKPGKAPKTLIYRANRLVDGVPSRFSGSGSGQDYTLTISSLQPEDFATYYCLQYDEFPLTFGGGTKVEIKRTVAAPSVFIFPPSDEQLKSGTASVVCLLNNFYPREAKVQWKVDNALQSGNSQESVTEQDSKDSTYSLSSTLTLSKADYEKHKVYACEVTHQGLSSPVTKSFNRGEC

SEQ ID NO: 13 - protein, 446 aa, synthetic construct
QVQLVQSGAEVKKPGSSVKVSCKASGYTFTDYNMHWVRQAPGQGLEWIGYIYPYNGGTGYNQKFKSKATITADESTNTAYMELSSLRSEDTAVYYCARGRPAMDYWGQGTLVTVSSASTKGPSVFPLAPSSKSTSGGTAALGCLVKDYFPEPVTVSWNSGALTSGVHTFPAVLQSSGLYSLSSVVTVPSSSLGTQTYICNVNHKPSNTKVDKKVEPKSCDKTHTCPPCPAPEAAGGPSVFLFPPKPKDTLMISRTPEVTCVVVDVSHEDPEVKFNWYVDGVEVHNAKTKPREEQYNSTYRVVSVLTVLHQDWLNGKEYKCKVSNKALAASIEKTISKAKGQPREPQVYTLPPSRDELTKNQVSLTCLVKGFYPSDIAVEWESNGQPENNYKTTPPVLDSDGSFFLYSKLTVDKSRWQQGNVFSCSVMHEALHNHYTQKSLSLSPGK

SEQ ID NO: 14 - protein, 218 aa, synthetic construct
DIQMTQSPSSLSASVGDRVTITCRASESVDNYGISFMNWFQQKPGKAPKLLIYAASNQGSGVPSRFSGSGSGTDFTLTISSLQPDDFATYYCQQSKEVPWTFGQGTKVEIKRTVAAPSVFIFPPSDEQLKSGTASVVCLLNNFYPREAKVQWKVDNALQSGNSQESVTEQDSKDSTYSLSSTLTLSKADYEKHKVYACEVTHQGLSSPVTKSFNRGEC

SEQ ID NO: 15 - protein, 448 aa, synthetic construct
QVQLQQPGAEVVKPGASVKMSCKASGYTFTSYYIHWIKQTPGQGLEWVGVIYPGNDDISYNQKFQGKATLTADKSSTTAYMQLSSLTSEDSAVYYCAREVRLRYFDVWGQGTTVTVSSASTKGPSVFPLAPSSKSTSGGTAALGCLVKDYFPEPVTVSWNSGALTSGVHTFPAVLQSSGLYSLSSVVTVPSSSLGTQTYICNVNHKPSNTKVDKKVEPKSCDKTHTCPPCPAPEAAGGPSVFLFPPKPKDTLMISRTPEVTCVVVDVSHEDPEVKFNWYVDGVEVHNAKTKPREEQYNSTYRVVSVLTVLHQDWLNGKEYKCKVSNKALAASIEKTISKAKGQPREPQVYTLPPSRDELTKNQVSLTCLVKGFYPSDIAVEWESNGQPENNYKTTPPVLDSDGSFFLYSKLTVDKSRWQQGNVFSCSVMHEALHNHYTQKSLSLSPGK

SEQ ID NO: 16 - protein, 219 aa, synthetic construct; identical to SEQ ID NO: 10

SEQ ID NO: 17 - protein, 450 aa, synthetic construct
QVQLVQSGAEVKKPGASVKVSCKASGYIFTSSIMHWVRQAPGQGLEWIGYIKPYNDGTKYNEKFKGRATLTSDRSTSTAYMELSSLRSEDTAVYYCAREGGNDYYDTMDYWGQGTLVTVSSASTKGPSVFPLAPSSKSTSGGTAALGCLVKDYFPEPVTVSWNSGALTSGVHTFPAVLQSSGLYSLSSVVTVPSSSLGTQTYICNVNHKPSNTKVDKKVEPKSCDKTHTCPPCPAPELLGGPSVFLFPPKPKDTLMISRTPEVTCVVVDVSHEDPEVKFNWYVDGVEVHNAKTKPREEQYNSTYRVVSVLTVLHQDWLNGKEYKCKVSNKALPAPIEKTISKAKGQPREPQVYTLPPSRDELTKNQVSLTCLVKGFYPSDIAVEWESNGQPENNYKTTPPVLDSDGSFFLYSKLTVDKSRWQQGNVFSCSVMHEALHNHYTQKSLCLSPG

SEQ ID NO: 18 - protein, 214 aa, synthetic construct
DIQMTQSPSSLSASVGDRVTITCRASQDINSYLSWFQQKPGKAPKTLIYRVNRLVDGVPSRFSGSGSGNDYTLTISSLQPEDFATYYCLQYDAFPYTFGQGTKVEIKRTVAAPSVFIFPPSDEQLKSGTASVVCLLNNFYPREAKVQWKVDNALQSGNSQESVTEQDSKDSTYSLSSTLTLSKADYEKHKVYACEVTHQGLSSPVTKSFNRGEC

SEQ ID NO: 19 - protein, 451 aa, synthetic construct
QVQLVQSGAEVKKPGSSVKVSCKASGGTFSNYWMHWVRQAPGQGLEWMGATYRGHSDTYYNQKFKGRVTITADKSTSTAYMELSSLRSEDTAVYYCARGAIYDGYDVLDNWGQGTLVTVSSASTKGPSVFPLAPSSKSTSGGTAALGCLVKDYFPEPVTVSWNSGALTSGVHTFPAVLQSSGLYSLSSVVTVPSSSLGTQTYICNVNHKPSNTKVDKKVEPKSCDKTHTCPPCPAPELLGGPSVFLFPPKPKDTLMISRTPEVTCVVVDVSHEDPEVKFNWYVDGVEVHNAKTKPREEQYNSTYRVVSVLTVLHQDWLNGKEYKCKVSNKALPAPIEKTISKAKGQPREPQVYTLPPSRDELTKNQVSLTCLVKGFYPSDIAVEWESNGQPENNYKTTPPVLDSDGSFFLYSKLTVDKSRWQQGNVFSCSVMHEALHNHYTQKSLSLSPGK

SEQ ID NO: 20 - protein, 214 aa, synthetic construct
DIQMTQSPSSLSASVGDRVTITCSASQDISNYLNWYQQKPGKAPKLLIYYTSNLHSGVPSRFSGSGSGTDFTLTISSLQPEDFATYYCQQYRKLPWTFGQGTKLEIKRTVAAPSVFIFPPSDEQLKSGTASVVCLLNNFYPREAKVQWKVDNALQSGNSQESVTEQDSKDSTYSLSSTLTLSKADYEKHKVYACEVTHQGLSSPVTKSFNRGEC

SEQ ID NO: 21 - protein, 10 aa, synthetic construct
GFNIKDTYIH

SEQ ID NO: 22 - protein, 17 aa, synthetic construct
RIYPTNGYTRYADSVKG

SEQ ID NO: 23 - protein, 11 aa, synthetic construct
WGGDGFYAMDY

SEQ ID NO: 24 - protein, 11 aa, synthetic construct
RASQDVNTAVA

SEQ ID NO: 25 - protein, 7 aa, synthetic construct
SASFLYS

SEQ ID NO: 26 - protein, 9 aa, synthetic construct
QQHYTTPPT

SEQ ID NO: 27 - protein, 10 aa, synthetic construct
GFTFTDYTMD

SEQ ID NO: 28 - protein, 17 aa, synthetic construct
DVNPNSGGSIYNQRFKG

SEQ ID NO: 29 - protein, 10 aa, synthetic construct
NLGPSFYFDY

SEQ ID NO: 30 - protein, 11 aa, synthetic construct
KASQDVSIGVA

SEQ ID NO: 31 - protein, 7 aa, synthetic construct
SASYRYT

SEQ ID NO: 32 - protein, 9 aa, synthetic construct
QQYYIYPYT

SEQ ID NO: 33 - protein, 5 aa, synthetic construct
DSNIH

SEQ ID NO: 34 - protein, 17 aa, synthetic construct
YIYPYNGGTDYNQKFKN

SEQ ID NO: 35 - protein, 7 aa, synthetic construct
GNPWLAY

SEQ ID NO: 36 - protein, 15 aa, synthetic construct
RASESLDNYGIRFLT

SEQ ID NO: 37 - protein, 8 aa, synthetic construct
AASNQGSG

SEQ ID NO: 38 - protein, 9 aa, synthetic construct
QQTKEVPWS

SEQ ID NO: 39 - protein, 5 aa, synthetic construct
DSNIH

SEQ ID NO: 40 - protein, 17 aa, synthetic construct
YIYPYNGGTDYNQKFKN

SEQ ID NO: 41 - protein, 7 aa, synthetic construct
GNPWLAY

SEQ ID NO: 42 - protein, 15 aa, synthetic construct
RASESLDNYGIRFLT

SEQ ID NO: 43 - protein, 8 aa, synthetic construct
AASNQGSG

SEQ ID NO: 44 - protein, 9 aa, synthetic construct
QQTKEVPWS

SEQ ID NO: 45 - protein, 5 aa, synthetic construct
SYYIH

SEQ ID NO: 46 - protein, 17 aa, synthetic construct
VIYPGNDDISYNQKFQG

SEQ ID NO: 47 - protein, 9 aa, synthetic construct
EVRLRYFDV

SEQ ID NO: 48 - protein, 17 aa, synthetic construct
KSSQSVFFSSSQKNYLA

SEQ ID NO: 49 - protein, 7 aa, synthetic construct
WASTRES

SEQ ID NO: 50 - protein, 8 aa, synthetic construct
HQYLSSRT

SEQ ID NO: 51 - protein, 5 aa, synthetic construct
NYDIN

SEQ ID NO: 52 - protein, 17 aa, synthetic construct
WIYPGDGSTKYNEKFKA

SEQ ID NO: 53 - protein, 8 aa, synthetic construct
GYEDAMDY

SEQ ID NO: 54 - protein, 11 aa, synthetic construct
KASQDINSYLS

SEQ ID NO: 55 - protein, 7 aa, synthetic construct
RANRLVD

SEQ ID NO: 56 - protein, 9 aa, synthetic construct
LQYDEFPLT

SEQ ID NO: 57 - protein, 5 aa, synthetic construct
DYNMH

SEQ ID NO: 58 - protein, 16 aa, synthetic construct
YIYPYNGGTGYNQKFK

SEQ ID NO: 59 - protein, 7 aa, synthetic construct
GRPAMDY

SEQ ID NO: 60 - protein, 15 aa, synthetic construct
RASESVDNYGISFMN

SEQ ID NO: 61 - protein, 7 aa, synthetic construct
AASNQGS

SEQ ID NO: 62 - protein, 9 aa, synthetic construct
QQSKEVPWT

SEQ ID NO: 63 - protein, 5 aa, synthetic construct
SYYIH

SEQ ID NO: 64 - protein, 17 aa, synthetic construct
VIYPGNDDISYNQKFQG

SEQ ID NO: 65 - protein, 9 aa, synthetic construct
EVRLRYFDV

SEQ ID NO: 66 - protein, 17 aa, synthetic construct
KSSQSVFFSSSQKNYLA

SEQ ID NO: 67 - protein, 7 aa, synthetic construct
WASTRES

SEQ ID NO: 68 - protein, 8 aa, synthetic construct
HQYLSSRT

SEQ ID NO: 69 - protein, 5 aa, synthetic construct
SSIMH

SEQ ID NO: 70 - protein, 17 aa, synthetic construct
YIKPYNDGTKYNEKFKG

SEQ ID NO: 71 - protein, 12 aa, synthetic construct
EGGNDYYDTMDY

SEQ ID NO: 72 - protein, 11 aa, synthetic construct
RASQDINSYLS

SEQ ID NO: 73 - protein, 7 aa, synthetic construct
RVNRLVD

SEQ ID NO: 74 - protein, 9 aa, synthetic construct
LQYDAFPYT

SEQ ID NO: 75 - protein, 5 aa, synthetic construct
NYWMH

SEQ ID NO: 76 - protein, 17 aa, synthetic construct
ATYRGHSDTYYNQKFKG

SEQ ID NO: 77 - protein, 12 aa, synthetic construct
GAIYDGYDVLDN

SEQ ID NO: 78 - protein, 11 aa, synthetic construct
SASQDISNYLN

SEQ ID NO: 79 - protein, 7 aa, synthetic construct
YTSNLHS

SEQ ID NO: 80 - protein, 9 aa, synthetic construct
QQYRKLPWT